European Patent Specification EP 3 713 564 B1, published November 15, 2023. Title: Novel compounds as mPGES-1 inhibitors. Applicant: Khondrion IP B.V. The sequence listing filed with the application follows.

SEQUENCE LISTING (12 sequences)

SEQ ID NO: 1 - DNA, 21 bp, Artificial Sequence
  Primer
gattgtactcgcacgggctac

SEQ ID NO: 2 - DNA, 20 bp, Artificial Sequence
  Primer
ggataaggttggaccgcact

SEQ ID NO: 3 - DNA, 20 bp, Artificial Sequence
  Primer
aggactctgctcacgaagga

SEQ ID NO: 4 - DNA, 20 bp, Artificial Sequence
  Primer
tgacatggattggaacagca

SEQ ID NO: 5 - DNA, 20 bp, Artificial Sequence
  Primer
agcacactgctggtcatcaa

SEQ ID NO: 6 - DNA, 20 bp, Artificial Sequence
  Primer
ctccacatctgggtcactcc

SEQ ID NO: 7 - DNA, 18 bp, Artificial Sequence
  Primer
gctggggctgtaccacac

SEQ ID NO: 8 - DNA, 20 bp, Artificial Sequence
  Primer
gattcacctccaccacctga

SEQ ID NO: 9 - DNA, 18 bp, Artificial Sequence
  Primer
ggtagagaccgccggagt

SEQ ID NO: 10 - DNA, 21 bp, Artificial Sequence
  Primer
tcgtaccactttgcagaagca

SEQ ID NO: 11 - DNA, 20 bp, Artificial Sequence
  Primer
agggtggtgactttacacgc

SEQ ID NO: 12 - DNA, 20 bp, Artificial Sequence
  Primer
gatgccaggacctgtatgct